European Patent Specification EP 3 446 102 B1, published December 10, 2025. Title: METHODS, SYSTEMS AND DEVICES FOR IN-PEN ASSAYS. Applicant: Berkeley Lights Inc. The sequence listing filed with the application follows.

SEQUENCE LISTING (11 sequences)

SEQ ID NO: 1 - protein, 20 aa, Artificial Sequence
  IgG binding peptide
  MISC_FEATURE (1)..(4): Xaa is any amino acid or absent
  MISC_FEATURE (5)..(5): Xaa is Cys or Ser
  MISC_FEATURE (6)..(11): Xaa is any amino acid
  MISC_FEATURE (16)..(20): Xaa is any amino acid or absent
XXXXXXXXXXXLVWCXXXXX

SEQ ID NO: 2 - protein, 20 aa, Artificial Sequence
  IgG binding peptide
  MISC_FEATURE (1)..(4): Xaa is any amino acid or absent
  MISC_FEATURE (5)..(5): Xaa is Cys or Ser
  MISC_FEATURE (6)..(9): Xaa is any amino acid
  MISC_FEATURE (16)..(20): Xaa is any amino acid or absent
XXXXXXXXXGELVWCXXXXX

SEQ ID NO: 3 - protein, 20 aa, Artificial Sequence
  IgG binding peptide
  MISC_FEATURE (1)..(4): Xaa is any amino acid or absent
  MISC_FEATURE (5)..(5): Xaa is Cys or Ser
  MISC_FEATURE (6)..(6): Xaa is Ala, Ser, or Thr
  MISC_FEATURE (7)..(7): Xaa is Trp or Tyr
  MISC_FEATURE (8)..(8): Xaa is His or Trp
  MISC_FEATURE (9)..(9): Xaa is Leu or Met
  MISC_FEATURE (16)..(20): Xaa is any amino acid or absent
XXXXXXXXXGELVWCXXXXX

SEQ ID NO: 4 - protein, 20 aa, Artificial Sequence
  IgG binding peptide
  MISC_FEATURE (1)..(3): Xaa is any amino acid or absent
  MISC_FEATURE (4)..(4): Xaa is Ser, Arg, or Asp
  MISC_FEATURE (5)..(5): Xaa is Cys or Ser
  MISC_FEATURE (6)..(6): Xaa is Ala, Ser, or Thr
  MISC_FEATURE (7)..(7): Xaa is Trp or Tyr
  MISC_FEATURE (8)..(8): Xaa is His or Trp
  MISC_FEATURE (9)..(9): Xaa is Leu or Met
  MISC_FEATURE (16)..(16): Xaa is Glu, Ser, Thr, or Val
  MISC_FEATURE (17)..(20): Xaa is any amino acid or absent
XXXXXXXXXGELVWCXXXXX

SEQ ID NO: 5 - protein, 13 aa, Artificial Sequence
  IgG binding peptide
  MISC_FEATURE (1)..(1): Xaa is any amino acid or absent
  MISC_FEATURE (2)..(2): Xaa is Cys or Ser
  MISC_FEATURE (3)..(8): Xaa is any amino acid
  MISC_FEATURE (13)..(13): Xaa is any amino acid or absent
XXXXXXXXLVWCX

SEQ ID NO: 6 - protein, 13 aa, Artificial Sequence
  IgG binding peptide
  MISC_FEATURE (1)..(1): Xaa is any amino acid or absent
  MISC_FEATURE (2)..(2): Xaa is Cys or Ser
  MISC_FEATURE (3)..(6): Xaa is any amino acid
  MISC_FEATURE (13)..(13): Xaa is any amino acid or absent
XXXXXXGELVWCX

SEQ ID NO: 7 - protein, 13 aa, Artificial Sequence
  IgG binding peptide
  MISC_FEATURE (1)..(1): Xaa is any amino acid or absent
  MISC_FEATURE (2)..(2): Xaa is Cys or Ser
  MISC_FEATURE (3)..(3): Xaa is Ala, Ser, or Thr
  MISC_FEATURE (4)..(4): Xaa is Trp or Tyr
  MISC_FEATURE (5)..(5): Xaa is His or Trp
  MISC_FEATURE (6)..(6): Xaa is Leu or Met
  MISC_FEATURE (13)..(13): Xaa is any amino acid or absent
XXXXXXGELVWCX

SEQ ID NO: 8 - protein, 13 aa, Artificial Sequence
  IgG binding peptide
  MISC_FEATURE (1)..(1): Xaa is Ser, Arg, or Asp
  MISC_FEATURE (2)..(2): Xaa is Cys or Ser
  MISC_FEATURE (3)..(3): Xaa is Ala, Ser or Thr
  MISC_FEATURE (4)..(4): Xaa is Trp or Tyr
  MISC_FEATURE (5)..(5): Xaa is His or Trp
  MISC_FEATURE (6)..(6): Xaa is Leu or Met
  MISC_FEATURE (13)..(13): Xaa is Glu, Ser, Thr, or Val
XXXXXXGELVWCX

SEQ ID NO: 9 - protein, 13 aa, Artificial Sequence
  IgG binding peptide
DSAWHLGELVWCT

SEQ ID NO: 10 - protein, 13 aa, Artificial Sequence
  IgG binding peptide
DCAWHLGELVWCT

SEQ ID NO: 11 - RNA, 23 nt, Artificial Sequence
  IgG binding aptamer
  misc_RNA (1)..(5): Phosphate
  misc_RNA (6)..(6): 2'-F-RNA Phosphate
  misc_RNA (7)..(7): Phosphate
  misc_RNA (8)..(11): 2'F-RNA Phosphate
  misc_RNA (12)..(19): Phosphate
  misc_RNA (20)..(23): 2'-F-RNA Phosphate
ggaggugcuccgaaarraacucc